European Patent Application EP 4 163 370 A1, published April 12, 2023. Title: Stabilization of Nucleic Acids in Biological Samples. Applicant: Axagarius GmbH & Co. KG. The sequence listing filed with the application follows.

SEQUENCE LISTING (6 sequences)

SEQ ID NO: 1 - DNA, 22 bp, arteficial
  misc_feature: CDV forward primer
ctgtcrgtaatcgagrattcga

SEQ ID NO: 2 - DNA, 23 bp, arteficial
  misc_feature: CDV reverse primer
gccgaaagaatatccccagttag

SEQ ID NO: 3 - DNA, 24 bp, arteficial
  misc_feature: CDV probe
atcttcgccagartcytcagtgct

SEQ ID NO: 4 - DNA, 22 bp, arteficial
  misc_feature: POX forward primer
gccagagatatcatagccgctc

SEQ ID NO: 5 - DNA, 29 bp, arteficial
  misc_feature: POX reverse primer
caacgactaactaatttggaaaaaaagat

SEQ ID NO: 6 - DNA, 34 bp, arteficial
  misc_feature: POX probe
ttttccaacctaaatagaacttcatcgttgcgtt